European Patent Application EP 4 279 595 A1, published November 22, 2023. Title: POLYNUCLEOTIDES AND EXPRESSION CASSETTES COMPRISING CODING SEQUENCES OF TOLUENE DIOXYGENASE, AND USES THEREOF. Applicant: Shanghai Shengping Medical Equipment Co., Ltd. Shanghai VastPro Technology Development Co., Ltd. The sequence listing filed with the application follows.

SEQUENCE LISTING (13 sequences)

SEQ ID NO: 1 - DNA, 3591 bp, Artificial Sequence
  polynucleotide encoding toluene dioxygenase
atgaaccagaccgacacctctccgatccgtctgcgtcgttcttggaacacctctgaaatcgaagctctgttcgacgaacacgctggtcgtatcgacccgcgtatctacaccgacgaagacctgtaccagctggaactcgaacgtgtcttcgcgcgttcttggctgctgctgggtcacgaaacccagatccgtaaaccgggtgactacatcaccacctacatgggtgaagacccggttgttgttgttcgtcagaaagacgcttctatcgctgttttcctgaaccagtgccgtcaccgtggtatgcgtatctgccgtgctgacgctggtaacgctaaagctttcacctgctcttaccacggttgggcttacgacaccgctggtaacctggttaacgttccgtacgaagctgaatctttcgcttgcctgaacaaaaaagaatggtctccgctgaaagctcgtgttgaaacctacaaaggtctgatcttcgctaactgggacgaaaacgctgttgacctggacacctacctgggtgaagctaaattctacatggaccacatgctggaccgtaccgaagctggtaccgaagctatcccgggtgttcagaaatgggttatcccgtgcaactggaaattcgctgctgaacagttctgctctgacatgtaccacgctggtaccacctctcacctgtctggtatcctggctggtctgccggaagacctggaaatggctgacctggctccgccgaccgttggtaaacagtaccgtgcttcttggggtggtcacggttctggtttctacgttggtgacccgaacctgatgctggctatcatgggtccgaaagttacctcttactggaccgaaggtccggcttctgaaaaagctgctgaacgtctgggttctgttgaacgtggttctaaactgatggttgaacacatgaccgttttcccgacctgctctttcctgccgggtatcaacaccgttcgtacctggcacccgcgtggtccgaacgaggttgaagtatgggcgttcaccgttgttgacgctgacgctccggacgacatcaaagaagaattccgtcgtcagaccctgcgtaccttctctgctggtggtgttttcgaacaggacgacggtgaaaactgggttgaaatccagcacatcctgcgtggtcacaaagctcgttctcgtccgttcaacgctgaaatgtctatggaccagaccgttgacaacgacccggtttacccgggtcgtatctctaacaacgtttactctgaagaagctgctcgtggtctgtacgctcactggctgcgtatgatgacctctccggactgggacgctctgaaagctacccgttaatcgagatctcgatcccgcgaaattaatacgactcactataggggaattgtgagcggataacaattcccctctagaaataattttgtttaactttaagaaggagatataccatgatcgactctgctaaccgtgctgacgttttcctgcgtaaaccggctccggttgctccggaactgcagcacgaagttgaacagttctactactgggaagctaaactgctgaacgaccgtcgtttcgaagaatggttcgctctgctggctgaagacatccactacttcatgccgatccgtaccacccgtatcatgcgtgactctcgtctggaatactctggttctcgtgaatacgctcacttcgacgacgacgctaccatgatgaaaggtcgtctgcgtaaaatcacctctgacgtttcttggtctgaaaacccggcttctcgtacccgtcacctggtttctaacgttatgatcgttggtgctgaagctgaaggtgaatacgaaatctcttctgctttcatcgtttaccgtaaccgtctggaacgtcagctggacatcttcgctggtgaacgtcgtgacaccctgcgtcgtaacacctctgaagctggtttcgaaatcgttaaccgtaccatcctgatcgaccagtctaccatcctggctaacaacctgtctttcttcttctaagtgatgtcatgacctggacctacatcctgcgtcagggtgacctgccgccgggtgaaatgcagcgttacgaaggtggtccggaaccggttatggtttgcaacgttgacggtgaatttttcgctgttcaggacacctgcacccacggtgactgggctctgtctgacggttacctggacggtgacatcgttgaatgcaccctgcacttcggtaaattctgcgttcgtaccggtaaagttaaagctctgccggcttgcaaaccgatcaaagttttcccgatcaaagttgaaggtgacgaagttcacgttgacctggacaacggtgaactgaaataatggctacccacgttgctatcatcggtaacggcgttggtggcttcaccaccgctcaggctctgcgtgcggaaggcttcgaaggtcgtatatctctgatcggtgacgaaccgcacctgccgtacgaccgtccgtctctgtctaaagctgttctggacggttctctggaacgtccgccgatcctggctgaagctgactggtacggtgaagctcgtatcgacatgctgaccggtccggaagttaccgctctggacgttcagacccgtaccatctctctggacgacggtaccaccctgtctgctgacgctatcgttatcgctaccggttctcgtgctcgtactatggctctgccgggttctcagctgccgggtgttgttaccctgcgtacctacggtgacgttcaggttctgcgtgactcttggacctctgctacccgtctgctgatcgttggtggtggtctgatcggttgcgaagttgctaccaccgctcgtaaactgggtctgtctgttaccatcctggaagctggtgacgaactgctggttcgtgttctgggtcgtcgtatcggtgcttggctgcgtggtctgctgaccgaactgggtgttcaggttgaactgggtaccggtgttgttggtttctctggtgaaggtcagctggaacaggttatggcttctgacggtcgttctttcgttgctgactctgctctgatctgcgttggtgctgaaccggctgaccagctggctcgtcaggctggtctggcttgcgaccgtggtgttatcgttgaccactgcggtgctaccctggctaaaggtgttttcgctgttggtgacgttgcttcttggccgctgcgtgctggtggtcgtcgttctctggaaacctacatgaacgctcagcgtcaggctgctgctgttgctgctgctatcctgggtaaaaacgtttctgcgccgcagctgccggtgagctggaccgaaatcgctggtcaccgtatgcagatggctggtgacatcgaaggtccgggtgacttcgtttctcgtggtatgccgggttctggtgctgctctgctgttccgtctgcaagaacgtcgtatccaggctgttgttgctgttgacgctccgcgtgacttcgctctggctacccgtctggttgaagctcgtgctgctatcgaaccggctcgtctggctgacctgtctaactctatgcgtgacttcgttcgtgctaacgaaggtgacctgacctaa

SEQ ID NO: 2 - DNA, 3597 bp, Artificial Sequence
  polynucleotide encoding toluene dioxygenase
atgaaccagaccgacacctctccgatccgtctgcgtcgttcttggaacacctctgaaatcgaagctctgttcgacgaacacgctggtcgtatcgacccgcgtatctacaccgacgaagacctgtaccagctggaactcgaacgtgtcttcgcgcgttcttggctgctgctgggtcacgaaacccagatccgtaaaccgggtgactacatcaccacctacatgggtgaagacccggttgttgttgttcgtcagaaagacgcttctatcgctgttttcctgaaccagtgccgtcaccgtggtatgcgtatctgccgtgctgacgctggtaacgctaaagctttcacctgctcttaccacggttgggcttacgacaccgctggtaacctggttaacgttccgtacgaagctgaatctttcgcttgcctgaacaaaaaagaatggtctccgctgaaagctcgtgttgaaacctacaaaggtctgatcttcgctaactgggacgaaaacgctgttgacctggacacctacctgggtgaagctaaattctacatggaccacatgctggaccgtaccgaagctggtaccgaagctatcccgggtgttcagaaatgggttatcccgtgcaactggaaattcgctgctgaacagttctgctctgacatgtaccacgctggtaccacctctcacctgtctggtatcctggctggtctgccggaagacctggaaatggctgacctggctccgccgaccgttggtaaacagtaccgtgcttcttggggtggtcacggttctggtttctacgttggtgacccgaacctgatgctggctatcatgggtccgaaagttacctcttactggaccgaaggtccggcttctgaaaaagctgctgaacgtctgggttctgttgaacgtggttctaaactgatggttgaacacatgaccgttttcccgacctgctctttcctgccgggtatcaacaccgttcgtacctggcacccgcgtggtccgaacgaggttgaagtatgggcgttcaccgttgttgacgctgacgctccggacgacatcaaagaagaattccgtcgtcagaccctgcgtaccttctctgctggtggtgttttcgaacaggacgacggtgaaaactgggttgaaatccagcacatcctgcgtggtcacaaagctcgttctcgtccgttcaacgctgaaatgtctatggaccagaccgttgacaacgacccggtttacccgggtcgtatctctaacaacgtttactctgaagaagctgctcgtggtctgtacgctcactggctgcgtatgatgacctctccggactgggacgctctgaaagctacccgttaatcgagatctcgatcccgcgaaattaatacgactcactataggggaattgtgagcggataacaattcccctctagaaataattttgtttaactttaagaaggagatataccatgatcgactctgctaaccgtgctgacgttttcctgcgtaaaccggctccggttgctccggaactgcagcacgaagttgaacagttctactactgggaagctaaactgctgaacgaccgtcgtttcgaagaatggttcgctctgctggctgaagacatccactacttcatgccgatccgtaccacccgtatcatgcgtgactctcgtctggaatactctggttctcgtgaatacgctcacttcgacgacgacgctaccatgatgaaaggtcgtctgcgtaaaatcacctctgacgtttcttggtctgaaaacccggcttctcgtacccgtcacctggtttctaacgttatgatcgttggtgctgaagctgaaggtgaatacgaaatctcttctgctttcatcgtttaccgtaaccgtctggaacgtcagctggacatcttcgctggtgaacgtcgtgacaccctgcgtcgtaacacctctgaagctggtttcgaaatcgttaaccgtaccatcctgatcgaccagtctaccatcctggctaacaacctgtctttcttcttctaagaaggagatataccatgacctggacctacatcctgcgtcagggtgacctgccgccgggtgaaatgcagcgttacgaaggtggtccggaaccggttatggtttgcaacgttgacggtgaatttttcgctgttcaggacacctgcacccacggtgactgggctctgtctgacggttacctggacggtgacatcgttgaatgcaccctgcacttcggtaaattctgcgttcgtaccggtaaagttaaagctctgccggcttgcaaaccgatcaaagttttcccgatcaaagttgaaggtgacgaagttcacgttgacctggacaacggtgaactgaaataatggctacccacgttgctatcatcggtaacggcgttggtggcttcaccaccgctcaggctctgcgtgcggaaggcttcgaaggtcgtatatctctgatcggtgacgaaccgcacctgccgtacgaccgtccgtctctgtctaaagctgttctggacggttctctggaacgtccgccgatcctggctgaagctgactggtacggtgaagctcgtatcgacatgctgaccggtccggaagttaccgctctggacgttcagacccgtaccatctctctggacgacggtaccaccctgtctgctgacgctatcgttatcgctaccggttctcgtgctcgtactatggctctgccgggttctcagctgccgggtgttgttaccctgcgtacctacggtgacgttcaggttctgcgtgactcttggacctctgctacccgtctgctgatcgttggtggtggtctgatcggttgcgaagttgctaccaccgctcgtaaactgggtctgtctgttaccatcctggaagctggtgacgaactgctggttcgtgttctgggtcgtcgtatcggtgcttggctgcgtggtctgctgaccgaactgggtgttcaggttgaactgggtaccggtgttgttggtttctctggtgaaggtcagctggaacaggttatggcttctgacggtcgttctttcgttgctgactctgctctgatctgcgttggtgctgaaccggctgaccagctggctcgtcaggctggtctggcttgcgaccgtggtgttatcgttgaccactgcggtgctaccctggctaaaggtgttttcgctgttggtgacgttgcttcttggccgctgcgtgctggtggtcgtcgttctctggaaacctacatgaacgctcagcgtcaggctgctgctgttgctgctgctatcctgggtaaaaacgtttctgcgccgcagctgccggtgagctggaccgaaatcgctggtcaccgtatgcagatggctggtgacatcgaaggtccgggtgacttcgtttctcgtggtatgccgggttctggtgctgctctgctgttccgtctgcaagaacgtcgtatccaggctgttgttgctgttgacgctccgcgtgacttcgctctggctacccgtctggttgaagctcgtgctgctatcgaaccggctcgtctggctgacctgtctaactctatgcgtgacttcgttcgtgctaacgaaggtgacctgacctaa

SEQ ID NO: 3 - DNA, 110 bp, Artificial Sequence
  first spacer sequence
tcgagatctcgatcccgcgaaattaatacgactcactataggggaattgtgagcggataacaattcccctctagaaataattttgtttaactttaagaaggagatatacc

SEQ ID NO: 4 - protein, 450 aa, Pseudomonas putida
  TodC1
MNQTDTSPIRLRRSWNTSEIEALFDEHAGRIDPRIYTDEDLYQLELERVFARSWLLLGHETQIRKPGDYITTYMGEDPVVVVRQKDASIAVFLNQCRHRGMRICRADAGNAKAFTCSYHGWAYDTAGNLVNVPYEAESFACLNKKEWSPLKARVETYKGLIFANWDENAVDLDTYLGEAKFYMDHMLDRTEAGTEAIPGVQKWVIPCNWKFAAEQFCSDMYHAGTTSHLSGILAGLPEDLEMADLAPPTVGKQYRASWGGHGSGFYVGDPNLMLAIMGPKVTSYWTEGPASEKAAERLGSVERGSKLMVEHMTVFPTCSFLPGINTVRTWHPRGPNEVEVWAFTVVDADAPDDIKEEFRRQTLRTFSAGGVFEQDDGENWVEIQHILRGHKARSRPFNAEMSMDQTVDNDPVYPGRISNNVYSEEAARGLYAHWLRMMTSPDWDALKATR

SEQ ID NO: 5 - protein, 187 aa, Pseudomonas putida
  TodC2
MIDSANRADVFLRKPAPVAPELQHEVEQFYYWEAKLLNDRRFEEWFALLAEDIHYFMPIRTTRIMRDSRLEYSGSREYAHFDDDATMMKGRLRKITSDVSWSENPASRTRHLVSNVMIVGAEAEGEYEISSAFIVYRNRLERQLDIFAGERRDTLRRNTSEAGFEIVNRTILIDQSTILANNLSFFF

SEQ ID NO: 6 - protein, 107 aa, Pseudomonas putida
  TodB
MTWTYILRQGDLPPGEMQRYEGGPEPVMVCNVDGEFFAVQDTCTHGDWALSDGYLDGDIVECTLHFGKFCVRTGKVKALPACKPIKVFPIKVEGDEVHVDLDNGELK

SEQ ID NO: 7 - protein, 410 aa, Pseudomonas putida [sequence omitted]

SEQ ID NO: 8 - DNA, 19 bp, Artificial Sequence
  T7 promoter
taatacgactcactatagg

SEQ ID NO: 9 - DNA, 14 bp, Artificial Sequence
  prokaryotic ribosome binding site
gaaggagatatacc

SEQ ID NO: 10 - DNA, 17 bp, Artificial Sequence
  Lac operator
ttgtgagcggataacaa

SEQ ID NO: 11 - DNA, 48 bp, Artificial Sequence
  T7 terminator
ctagcataaccccttggggcctctaaacgggtcttgaggggttttttg

SEQ ID NO: 12 - DNA, 3591 bp, Pseudomonas putida
  nucleotides at positions 620-4210 in J04996.1
atgaatcagaccgacacatcacctatcaggctgcgcaggagctggaacaccagcgagatagaagcgctctttgacgagcatgccggacgtatcgatccgcgcatttataccgatgaggatctgtaccaactcgaactggagcgtgtcttcgcccggtcctggctgctgttggggcatgaaacccagattcgcaagccgggcgattacatcacgacctacatgggtgaagaccctgtcgtggtcgtccggcagaaagacgccagcattgccgtgttcctgaaccagtgccgccaccgtggcatgcgcatctgccgcgcggatgccggaaacgcgaaggcgttcacttgcagctaccacgggtgggcttacgacaccgccggcaatcttgtcaatgtgccttacgaggccgaatccttcgcgtgcctgaacaagaaggaatggagcccgctgaaggcccgggtagaaacctacaagggcctgattttcgccaactgggatgagaacgctgtagacctcgacacgtatctgggcgaggcgaagttctacatggaccacatgctcgaccgcaccgaggccggcaccgaagcgatcccgggcgtgcagaagtgggtcattccctgtaactggaaattcgccgcagagcagttttgcagcgacatgtaccatgccgggacgacctcgcatctgtctggcatcctggcaggcctgccagaagaccttgaaatggccgaccttgctccgccgacagttggcaagcagtaccgtgcgtcatggggcggacatggaagtggcttctatgtcggcgaccccaatctgatgcttgccatcatggggccaaaggtcaccagctactggaccgaaggccccgcgtcggaaaaggcggccgaacgtctgggtagcgtggagcgcggctcgaaactcatggtcgagcacatgaccgtcttccccacgtgttccttcctcccaggtatcaatacggtccggacatggcatccgcgcgggccgaacgaggtcgaggtatgggcgtttacggtggtcgatgctgatgctcctgacgatatcaaggaagagttccggcgccagacgctgcgcaccttctctgccggtggcgtgttcgagcaggacgacggggagaactgggtcgagatccagcacatcctgcgaggccacaaggcgcggagccgccctttcaatgccgagatgagcatggaccagaccgtcgacaacgacccggtttaccccgggcggatcagcaacaacgtctacagcgaggaagctgcccgcgggctctatgcccattggctgcggatgatgacatcccccgactgggacgcgctgaaggcgacacgctgaatccagagacagcttgcgccacgcagtggcgccggccagaggccgcatttgacttcgacccaggttggatgcggtggaccttgtccatttgaaatctacaaggaacgaccatgattgattcagccaacagagccgacgtctttctccgcaagccggcacccgtagcgcccgaactgcagcacgaagtcgagcagttctactattgggaggccaagcttctcaacgatcgccgcttcgaggagtggttcgcgctgctcgcggaagacattcactacttcatgcccattcgcaccacgcggatcatgcgggactcgcgccttgaatactcaggctcccgagagtacgcgcacttcgatgacgacgccacgatgatgaagggacgcttgcgcaagatcacgtccgacgtgagctggtccgagaaccccgcatcgcggacccggcatctcgtgagcaacgtgatgatcgtcggcgcagaggcagaaggggagtacgaaatctcaagcgccttcattgtgtaccgcaatcgtctggagcggcagctcgacatctttgccggtgagcgtcgcgatacgttgcgccgtaacacgagcgaggccgggttcgagatcgtcaatcggaccatcctgatcgaccagagcaccatcctggccaataacctcagtttcttcttctaggtgatgtcatgacttggacatacatattgcggcagggtgacctgccacccggtgagatgcagcgctacgaaggcggcccggaacctgtgatggtctgcaacgtcgatggcgagttcttcgcggtgcaggatacctgcacgcatggggactgggcgttgtcggatggttacctggacggtgatattgtcgaatgcacgttgcatttcggcaagttctgcgtgcggaccgggaaggtgaaggcgctgcctgcttgcaaacctatcaaggtattcccaatcaaggtcgaaggcgatgaagtgcacgtcgatctcgacaacggggagttgaagtgatggctacccatgtggcgatcatcggcaatggcgtgggtggcttcacgaccgcgcaggccctacgtgccgagggcttcgaggggagaatctcgctgattggggacgaaccgcatctcccctatgaccgaccatccttgtccaaggcggttctcgacggcagccttgagcggccgcccatactggccgaggccgattggtacggcgaggcccgcatcgacatgctgaccggcccggaagtcactgcccttgatgtgcagacaaggacgatcagtctggatgatggcaccacgctctctgcggacgccatcgtcatcgcgacgggcagtcgagcgcggacgatggcgttgcccggcagccaactgcccggcgtcgtaacgctgcgcacctacggtgacgtgcaggtattgcgcgatagttggacttccgcgacgcggctgctgattgtgggtggcggattgatcggctgcgaggtcgcgacgacggcgcgcaagctcggcctgtcggtcacgatcctggaggcaggtgatgaactgctggtccgagtacttgggcggcgtatcggtgcctggctgcgcggcctgctgacagaacttggtgtgcaggtcgagttgggaacgggtgtcgtaggtttttctggtgagggccagctcgaacaagtcatggccagcgatgggcgcagcttcgtagccgatagcgcactcatttgcgtcggcgcggagcccgcggatcaacttgcgcgtcaagcgggcttggcatgtgaccgcggcgtcattgtcgatcactgcggtgcgacgcttgccaaaggcgtattcgccgtcggagatgtggccagttggccgctgcgcgccggcggccggcgttcgctcgaaacctatatgaacgcgcagcgccaagccgccgcggtggctgcggccattctggggaaaaacgtatcggcaccgcaactgcccgtgtcctggacggagatcgctgggcatcgcatgcagatggcgggcgatatcgaaggacctggtgatttcgtctcgcgcggcatgcccggtagtggcgctgccctgttgttccgcctgcaggagcgaaggattcaggcggtcgtcgcggtcgatgcaccccgtgacttcgcgcttgcaacccgattggtagaagcccgcgcggcaatcgagccagcacggctggcagatctttcaaacagtatgcgcgattttgttcgtgcgaatgaaggagacctaacgtga

SEQ ID NO: 13 - DNA, 3590 bp, Artificial Sequence
  polynucleotide encoding toluene dioxygenase
atgaaccagaccgacacctctccgatccgtctgcgtcgttcttggaacacctctgaaatcgaagctctgttcgacgaacacgctggtcgtatcgacccgcgtatctacaccgacgaagacctgtaccagctggaactcgaacgtgtcttcgcgcgttcttggctgctgctgggtcacgaaacccagatccgtaaaccgggtgactacatcaccacctacatgggtgaagacccggttgttgttgttcgtcagaaagacgcttctatcgctgttttcctgaaccagtgccgtcaccgtggtatgcgtatctgccgtgctgacgctggtaacgctaaagctttcacctgctcttaccacggttgggcttacgacaccgctggtaacctggttaacgttccgtacgaagctgaatctttcgcttgcctgaacaaaaaagaatggtctccgctgaaagctcgtgttgaaacctacaaaggtctgatcttcgctaactgggacgaaaacgctgttgacctggacacctacctgggtgaagctaaattctacatggaccacatgctggaccgtaccgaagctggtaccgaagctatcccgggtgttcagaaatgggttatcccgtgcaactggaaattcgctgctgaacagttctgctctgacatgtaccacgctggtaccacctctcacctgtctggtatcctggctggtctgccggaagacctggaaatggctgacctggctccgccgaccgttggtaaacagtaccgtgcttcttggggtggtcacggttctggtttctacgttggtgacccgaacctgatgctggctatcatgggtccgaaagttacctcttactggaccgaaggtccggcttctgaaaaagctgctgaacgtctgggttctgttgaacgtggttctaaactgatggttgaacacatgaccgttttcccgacctgctctttcctgccgggtatcaacaccgttcgtacctggcacccgcgtggtccgaacgaggttgaagtatgggcgttcaccgttgttgacgctgacgctccggacgacatcaaagaagaattccgtcgtcagaccctgcgtaccttctctgctggtggtgttttcgaacaggacgacggtgaaaactgggttgaaatccagcacatcctgcgtggtcacaaagctcgttctcgtccgttcaacgctgaaatgtctatggaccagaccgttgacaacgacccggtttacccgggtcgtatctctaacaacgtttactctgaagaagctgctcgtggtctgtacgctcactggctgcgtatgatgacctctccggactgggacgctctgaaagctacccgttaatccagagacagcttgcgccacgcagtggcgccggccagaggccgcatttgacttcgacccaggttggatgcggtggaccttgtccatttgaaatctacaaggaacgaccatgatcgactctgctaaccgtgctgacgttttcctgcgtaaaccggctccggttgctccggaactgcagcacgaagttgaacagttctactactgggaagctaaactgctgaacgaccgtcgtttcgaagaatggttcgctctgctggctgaagacatccactacttcatgccgatccgtaccacccgtatcatgcgtgactctcgtctggaatactctggttctcgtgaatacgctcacttcgacgacgacgctaccatgatgaaaggtcgtctgcgtaaaatcacctctgacgtttcttggtctgaaaacccggcttctcgtacccgtcacctggtttctaacgttatgatcgttggtgctgaagctgaaggtgaatacgaaatctcttctgctttcatcgtttaccgtaaccgtctggaacgtcagctggacatcttcgctggtgaacgtcgtgacaccctgcgtcgtaacacctctgaagctggtttcgaaatcgttaaccgtaccatcctgatcgaccagtctaccatcctggctaacaacctgtctttcttcttctaagtgatgtcatgacctggacctacatcctgcgtcagggtgacctgccgccgggtgaaatgcagcgttacgaaggtggtccggaaccggttatggtttgcaacgttgacggtgaatttttcgctgttcaggacacctgcacccacggtgactgggctctgtctgacggttacctggacggtgacatcgttgaatgcaccctgcacttcggtaaattctgcgttcgtaccggtaaagttaaagctctgccggcttgcaaaccgatcaaagttttcccgatcaaagttgaaggtgacgaagttcacgttgacctggacaacggtgaactgaaataatggctacccacgttgctatcatcggtaacggcgttggtggcttcaccaccgctcaggctctgcgtgcggaaggcttcgaaggtcgtatatctctgatcggtgacgaaccgcacctgccgtacgaccgtccgtctctgtctaaagctgttctggacggttctctggaacgtccgccgatcctggctgaagctgactggtacggtgaagctcgtatcgacatgctgaccggtccggaagttaccgctctggacgttcagacccgtaccatctctctggacgacggtaccaccctgtctgctgacgctatcgttatcgctaccggttctcgtgctcgtactatggctctgccgggttctcagctgccgggtgttgttaccctgcgtacctacggtgacgttcaggttctgcgtgactcttggacctctgctacccgtctgctgatcgttggtggtggtctgatcggttgcgaagttgctaccaccgctcgtaaactgggtctgtctgttaccatcctggaagctggtgacgaactgctggttcgtgttctgggtcgtcgtatcggtgcttggctgcgtggtctgctgaccgaactgggtgttcaggttgaactgggtaccggtgttgttggtttctctggtgaaggtcagctggaacaggttatggcttctgacggtcgttctttcgttgctgactctgctctgatctgcgttggtgctgaaccggctgaccagctggctcgtcaggctggtctggcttgcgaccgtggtgttatcgttgaccactgcggtgctaccctggctaaaggtgttttcgctgttggtgacgttgcttcttggccgctgcgtgctggtggtcgtcgttctctggaaacctacatgaacgctcagcgtcaggctgctgctgttgctgctgctatcctgggtaaaaacgtttctgcgccgcagctgccggtgagctggaccgaaatcgctggtcaccgtatgcagatggctggtgacatcgaaggtccgggtgacttcgtttctcgtggtatgccgggttctggtgctgctctgctgttccgtctgcaagaacgtcgtatccaggctgttgttgctgttgacgctccgcgtgacttcgctctggctacccgtctggttgaagctcgtgctgctatcgaaccggctcgtctggctgacctgtctaactctatgcgtgacttcgttcgtgctaacgaaggtgacctgacctaa